European Patent Specification EP 3 738 599 B1, published December 27, 2023. Title: COMPOSITION COMPRISING PROBIOTICS AND POLYPEPTIDE HAVING BINDING AFFINITY FOR IGE AND USE THEREOF. Applicant: PROGEN CO., LTD. GI INNOVATION, INC. Application 19738433.2. The sequence listing filed with the application follows.

SEQUENCE LISTING (22 sequences)

SEQ ID NO: 1 - protein, 180 aa, Artificial Sequence
  FCeRI1 ECD
VPQKPKVSLNPPWNRIFKGENVTLTCNGNNFFEVSSTKWFHNGSLSEETNSSLNIVNAKFEDSGEYKCQHQQVNESEPVYLEVFSDWLLLQASAEVVMEGQPLFLRCHGWRNWDVYKVIYYKDGEALKYWYENHNISITNATVEDSGTYYCTGKVWQLDYESEPLNITVIKAPREKYWLQ

SEQ ID NO: 2 - protein, 215 aa, Artificial Sequence
  Modified Fc
SHTQPLGVFLFPPKPKDTLMISRTPEVTCVVVDVSQEDPEVQFNWYVDGVEVHNAKTKPREEQFNSTYRVVSVLTVLHQDWLNGKEYKCKVSNKGLPSSIEKTISKAKGQPREPQVYTLPPSQEEMTKNQVSLTCLVKGFYPSDIAVEWESNGQPENNYKTTPPVLDSDGSFFLYSRLTVDKSRWQEGNVFSCSVMHEALHNHYTQKSLSLSLGK

SEQ ID NO: 3 - protein, 30 aa, Artificial Sequence
  IgD hinge variant
RNTGRGGEEKKGSKEKEEQEERETKTPECP

SEQ ID NO: 4 - protein, 49 aa, Artificial Sequence
  IgD hinge variant
AQPQAEGSLAKATTAPATTRNTGRGGEEKKGSKEKEEQEERETKTPECP

SEQ ID NO: 5 - DNA, 540 bp, Artificial Sequence
  nucleotides sequence of FCeRI1 ECD
gtgccccagaagcccaaggtgagcctgaaccctccctggaacagaatcttcaagggcgagaacgtgaccctgacctgcaacggcaacaacttcttcgaggtgagcagcaccaagtggttccacaatggcagcctgagcgaggagaccaacagctccctgaacatcgtgaacgccaagttcgaggacagcggcgagtacaagtgccagcaccagcaggtgaacgagagcgagcccgtgtacctggaggtgttcagcgactggctgctgctgcaggccagcgccgaggtggtgatggagggccagcccctgttcctgagatgccacggctggagaaactgggacgtgtacaaggtgatctactacaaggatggcgaggccctgaagtactggtacgagaaccacaacatctccatcaccaacgccaccgtggaggacagcggcacctactactgcacaggcaaggtgtggcagctggactacgagagcgagcccctgaacatcaccgtgatcaaggctcccagagagaagtactggctgcag

SEQ ID NO: 6 - DNA, 561 bp, Artificial Sequence
  nucleotides sequence of modified Fc
tgcgtggtcgtggatgtgagccaggaagatcccgaagtgcagttcaactggtacgtggatggcgtggaagtgcacaacgccaagaccaagcccagagaagagcagttcaactccacctacagagtggtgagcgtgctgaccgtgctgcaccaggactggctgaacggcaaggagtacaagtgcaaggtgtccaacaaaggcctgcccagctccatcgagaagaccatcagcaaagccaaaggccagcccagagaaccccaggtgtacaccctgcctcccagccaggaagagatgaccaagaaccaggtgtccctgacctgcctggtgaaaggcttctaccccagcgacatcgccgtggagtgggaaagcaacggccagcccgagaacaattacaagacaacccctcccgtgctggatagcgatggcagcttctttctgtacagcagactgaccgtggacaagagcagatggcaggaaggcaacgtgttcagctgcagcgtgatgcacgaagccctgcacaaccactacacccagaagagcctgtccctgagcctgggcaag

SEQ ID NO: 7 - DNA, 174 bp, Artificial Sequence
  nucleotides sequence of IgD hinge variant
aggaacaccggcagaggaggcgaggaaaagaaaggaagcaaggagaaggaggagcaggaggaaagagaaaccaagacccccgagtgccccagccacacccagcccctgggcgtgttcctgttcccccccaagcccaaggacaccctgatgatcagcagaacccccgaggtgacc

SEQ ID NO: 8 - DNA, 231 bp, Artificial Sequence
  nucleotides sequence of IgD hinge variant
gcccagccccaggccgagggcagcctggctaaggccaccacagctcccgccaccaccaggaacaccggcagaggaggcgaggaaaagaaaggaagcaaggagaaggaggagcaggaggaaagagaaaccaagacccccgagtgccccagccacacccagcccctgggcgtgttcctgttcccccccaagcccaaggacaccctgatgatcagcagaacccccgaggtgacc

SEQ ID NO: 9 - protein, 25 aa, Artificial Sequence
  signal peptide
MDAMLRGLCCVLLLCGAVFVSPSHA

SEQ ID NO: 10 - DNA, 75 bp, Artificial Sequence
  nucleotides sequence of signal peptide
atggacgccatgctgagaggcctgtgctgtgtgctgctgctgtgcggcgccgtgttcgtgtcccctagccacgcc

SEQ ID NO: 11 - protein, 450 aa, Artificial Sequence
  FceRIa ECD-hinge-Fc2
MDAMLRGLCCVLLLCGAVFVSPSHAVPQKPKVSLNPPWNRIFKGENVTLTCNGNNFFEVSSTKWFHNGSLSEETNSSLNIVNAKFEDSGEYKCQHQQVNESEPVYLEVFSDWLLLQASAEVVMEGQPLFLRCHGWRNWDVYKVIYYKDGEALKYWYENHNISITNATVEDSGTYYCTGKVWQLDYESEPLNITVIKAPREKYWLQRNTGRGGEEKKGSKEKEEQEERETKTPECPSHTQPLGVFLFPPKPKDTLMISRTPEVTCVVVDVSQEDPEVQFNWYVDGVEVHNAKTKPREEQFNSTYRVVSVLTVLHQDWLNGKEYKCKVSNKGLPSSIEKTISKAKGQPREPQVYTLPPSQEEMTKNQVSLTCLVKGFYPSDIAVEWESNGQPENNYKTTPPVLDSDGSFFLYSRLTVDKSRWQEGNVFSCSVMHEALHNHYTQKSLSLSLGK

SEQ ID NO: 12 - DNA, 1350 bp, Artificial Sequence
  nucleotides sequence of FceRIa ECD-hinge-Fc2
atggacgccatgctgagaggcctgtgctgtgtgctgctgctgtgcggcgccgtgttcgtgtcccctagccacgccgtgccccagaagcccaaggtgagcctgaaccctccctggaacagaatcttcaagggcgagaacgtgaccctgacctgcaacggcaacaacttcttcgaggtgagcagcaccaagtggttccacaatggcagcctgagcgaggagaccaacagctccctgaacatcgtgaacgccaagttcgaggacagcggcgagtacaagtgccagcaccagcaggtgaacgagagcgagcccgtgtacctggaggtgttcagcgactggctgctgctgcaggccagcgccgaggtggtgatggagggccagcccctgttcctgagatgccacggctggagaaactgggacgtgtacaaggtgatctactacaaggatggcgaggccctgaagtactggtacgagaaccacaacatctccatcaccaacgccaccgtggaggacagcggcacctactactgcacaggcaaggtgtggcagctggactacgagagcgagcccctgaacatcaccgtgatcaaggctcccagagagaagtactggctgcagaggaacaccggcagaggaggcgaggaaaagaaaggaagcaaggagaaggaggagcaggaggaaagagaaaccaagacccccgagtgccccagccacacccagcccctgggcgtgttcctgttcccccccaagcccaaggacaccctgatgatcagcagaacccccgaggtgacctgcgtggtcgtggatgtgagccaggaagatcccgaagtgcagttcaactggtacgtggatggcgtggaagtgcacaacgccaagaccaagcccagagaagagcagttcaactccacctacagagtggtgagcgtgctgaccgtgctgcaccaggactggctgaacggcaaggagtacaagtgcaaggtgtccaacaaaggcctgcccagctccatcgagaagaccatcagcaaagccaaaggccagcccagagaaccccaggtgtacaccctgcctcccagccaggaagagatgaccaagaaccaggtgtccctgacctgcctggtgaaaggcttctaccccagcgacatcgccgtggagtgggaaagcaacggccagcccgagaacaattacaagacaacccctcccgtgctggatagcgatggcagcttctttctgtacagcagactgaccgtggacaagagcagatggcaggaaggcaacgtgttcagctgcagcgtgatgcacgaagccctgcacaaccactacacccagaagagcctgtccctgagcctgggcaag

SEQ ID NO: 13 - protein, 469 aa, Artificial Sequence
  FceRIa ECD-hinge-Fc3
MDAMLRGLCCVLLLCGAVFVSPSHAVPQKPKVSLNPPWNRIFKGENVTLTCNGNNFFEVSSTKWFHNGSLSEETNSSLNIVNAKFEDSGEYKCQHQQVNESEPVYLEVFSDWLLLQASAEVVMEGQPLFLRCHGWRNWDVYKVIYYKDGEALKYWYENHNISITNATVEDSGTYYCTGKVWQLDYESEPLNITVIKAPREKYWLQAQPQAEGSLAKATTAPATTRNTGRGGEEKKGSKEKEEQEERETKTPECPSHTQPLGVFLFPPKPKDTLMISRTPEVTCVVVDVSQEDPEVQFNWYVDGVEVHNAKTKPREEQFNSTYRVVSVLTVLHQDWLNGKEYKCKVSNKGLPSSIEKTISKAKGQPREPQVYTLPPSQEEMTKNQVSLTCLVKGFYPSDIAVEWESNGQPENNYKTTPPVLDSDGSFFLYSRLTVDKSRWQEGNVFSCSVMHEALHNHYTQKSLSLSLGK

SEQ ID NO: 14 - DNA, 1407 bp, Artificial Sequence
  nucleotides sequence of FceRIa ECD-hinge-Fc3
atggacgccatgctgagaggcctgtgctgtgtgctgctgctgtgcggcgccgtgttcgtgtcccctagccacgccgtgccccagaagcccaaggtgagcctgaaccctccctggaacagaatcttcaagggcgagaacgtgaccctgacctgcaacggcaacaacttcttcgaggtgagcagcaccaagtggttccacaatggcagcctgagcgaggagaccaacagctccctgaacatcgtgaacgccaagttcgaggacagcggcgagtacaagtgccagcaccagcaggtgaacgagagcgagcccgtgtacctggaggtgttcagcgactggctgctgctgcaggccagcgccgaggtggtgatggagggccagcccctgttcctgagatgccacggctggagaaactgggacgtgtacaaggtgatctactacaaggatggcgaggccctgaagtactggtacgagaaccacaacatctccatcaccaacgccaccgtggaggacagcggcacctactactgcacaggcaaggtgtggcagctggactacgagagcgagcccctgaacatcaccgtgatcaaggctcccagagagaagtactggctgcaggcccagccccaggccgagggcagcctggctaaggccaccacagctcccgccaccaccaggaacaccggcagaggaggcgaggaaaagaaaggaagcaaggagaaggaggagcaggaggaaagagaaaccaagacccccgagtgccccagccacacccagcccctgggcgtgttcctgttcccccccaagcccaaggacaccctgatgatcagcagaacccccgaggtgacctgcgtggtcgtggatgtgagccaggaagatcccgaagtgcagttcaactggtacgtggatggcgtggaagtgcacaacgccaagaccaagcccagagaagagcagttcaactccacctacagagtggtgagcgtgctgaccgtgctgcaccaggactggctgaacggcaaggagtacaagtgcaaggtgtccaacaaaggcctgcccagctccatcgagaagaccatcagcaaagccaaaggccagcccagagaaccccaggtgtacaccctgcctcccagccaggaagagatgaccaagaaccaggtgtccctgacctgcctggtgaaaggcttctaccccagcgacatcgccgtggagtgggaaagcaacggccagcccgagaacaattacaagacaacccctcccgtgctggatagcgatggcagcttctttctgtacagcagactgaccgtggacaagagcagatggcaggaaggcaacgtgttcagctgcagcgtgatgcacgaagccctgcacaaccactacacccagaagagcctgtccctgagcctgggcaag

SEQ ID NO: 15 - protein, 406 aa, Artificial Sequence
  human a-2,6 sialic acid transferase
MIHTNLKKKFSCCVLVFLLFAVICVWKEKKKGSYYDSFKLQTKEFQVLKSLGKLAMGSDSQSVSSSSTQDPHRGRQTLGSLRGLAKAKPEASFQVWNKDSSSKNLIPRLQKIWKNYLSMNKYKVSYKGPGPGIKFSAEALRCHLRDHVNVSMVEVTDFPFNTSEWEGYLPKESIRTKAGPWGRCAVVSSAGSLKSSQLGREIDDHDAVLRFNGAPTANFQQDVGTKTTIRLMNSQLVTTEKRFLKDSLYNEGILIVWDPSVYHSDIPKWYQNPDYNFFNNYKTYRKLHPNQPFYILKPQMPWELWDILQEISPEEIQPNPPSSGMLGIIIMMTLCDQVDIYEFLPSKRKTDVCYYYQKFFDSACTMGAYHPLLYEKNLVKHLNQGTDEDIYLLGKATLPGFRTIHC

SEQ ID NO: 16 - DNA, 1218 bp, Artificial Sequence
  nucleotides sequence of human a-2,6 sialic acid transferase
atgatccacaccaacctgaagaagaagttcagctgctgcgtgctggtgttcctgctgttcgccgtgatctgcgtgtggaaggagaagaagaaaggcagctactacgacagcttcaagctgcagaccaaggagttccaggtgctgaagagcctgggcaagctggccatgggcagcgacagccagagcgtgtccagctcctccacccaggatccccacagaggcagacagaccctgggcagcctgagaggcctggccaaggccaagcccgaggccagcttccaggtgtggaacaaggacagcagcagcaagaacctgatccccagactgcagaagatctggaagaactacctgagcatgaacaagtacaaggtgagctacaaaggacccggacccggcatcaagttcagcgccgaggccctgaggtgccacctgagagaccacgtgaacgtgagcatggtggaagtgaccgacttccccttcaacaccagcgagtgggaaggctacctgcccaaggagagcatcaggaccaaggctggcccctggggcagatgcgccgtggtgagcagcgctggcagcctgaagagctcccagctgggcagagagatcgacgaccacgatgccgtgctgaggttcaatggcgctcccaccgccaacttccagcaggacgtgggcaccaagaccacaatccggctgatgaacagccagctggtgacaaccgagaagcggttcctgaaggacagcctgtacaacgagggcatcctgatcgtgtgggatcccagcgtgtaccacagcgacatccccaagtggtaccagaatcccgactacaacttcttcaacaactacaagacctatagaaagctgcaccccaaccagcccttctacatcctgaagccccagatgccctgggagctgtgggacatcctgcaggagatcagccctgaagagatccagcccaaccctccctccagcggcatgctgggcattatcatcatgatgaccctgtgcgaccaggtggacatctacgagttcctgcccagcaagagaaagaccgacgtgtgctactactatcagaagttcttcgacagcgcctgcaccatgggcgcctaccaccccctgctgtacgagaagaacctggtgaagcacctgaaccagggcaccgacgaggacatctacctgctgggcaaagccaccctgcccggcttcagaaccatccactgc

SEQ ID NO: 17 - protein, 30 aa, Artificial Sequence
  IgD hinge variant
  VARIANT (12)..(12): Xaa is selected from the group consisting of Lys and Gly.
  VARIANT (13)..(13): Xaa is selected from the group consisting of Glu, Gly and Ser.
RNTGRGGEEKKXXKEKEEQEERETKTPECP

SEQ ID NO: 18 - protein, 49 aa, Artificial Sequence
  IgD hinge variant
  VARIANT (31)..(31): Xaa is selected from the group consisting of Lys and Gly.
  VARIANT (32)..(32): Xaa is selected from the group consisting of Glu, Gly or Ser.
AQPQAEGSLAKATTAPATTRNTGRGGEEKKXXKEKEEQEERETKTPECP

SEQ ID NO: 19 - protein, 30 aa, Artificial Sequence
  IgD hinge
RNTGRGGEEKKKEKEKEEQEERETKTPECP

SEQ ID NO: 20 - protein, 425 aa, Artificial Sequence
  FceRIa ECD-hinge-Fc1
VPQKPKVSLNPPWNRIFKGENVTLTCNGNNFFEVSSTKWFHNGSLSEETNSSLNIVNAKFEDSGEYKCQHQQVNESEPVYLEVFSDWLLLQASAEVVMEGQPLFLRCHGWRNWDVYKVIYYKDGEALKYWYENHNISITNATVEDSGTYYCTGKVWQLDYESEPLNITVIKAPREKYWLQRNTGRGGEEKKKEKEKEEQEERETKTPECPSHTQPLGVFLFPPKPKDTLMISRTPEVTCVVVDVSQEDPEVQFNWYVDGVEVHNAKTKPREEQFNSTYRVVSVLTVLHQDWLNGKEYKCKVSNKGLPSSIEKTISKAKGQPREPQVYTLPPSQEEMTKNQVSLTCLVKGFYPSDIAVEWESNGQPENNYKTTPPVLDSDGSFFLYSRLTVDKSRWQEGNVFSCSVMHEALHNHYTQKSLSLSLGK

SEQ ID NO: 21 - protein, 425 aa, Artificial Sequence
  FceRIa ECD-hinge-Fc2
VPQKPKVSLNPPWNRIFKGENVTLTCNGNNFFEVSSTKWFHNGSLSEETNSSLNIVNAKFEDSGEYKCQHQQVNESEPVYLEVFSDWLLLQASAEVVMEGQPLFLRCHGWRNWDVYKVIYYKDGEALKYWYENHNISITNATVEDSGTYYCTGKVWQLDYESEPLNITVIKAPREKYWLQRNTGRGGEEKKGSKEKEEQEERETKTPECPSHTQPLGVFLFPPKPKDTLMISRTPEVTCVVVDVSQEDPEVQFNWYVDGVEVHNAKTKPREEQFNSTYRVVSVLTVLHQDWLNGKEYKCKVSNKGLPSSIEKTISKAKGQPREPQVYTLPPSQEEMTKNQVSLTCLVKGFYPSDIAVEWESNGQPENNYKTTPPVLDSDGSFFLYSRLTVDKSRWQEGNVFSCSVMHEALHNHYTQKSLSLSLGK

SEQ ID NO: 22 - protein, 444 aa, Artificial Sequence
  FceRIa ECD-hinge-Fc3
VPQKPKVSLNPPWNRIFKGENVTLTCNGNNFFEVSSTKWFHNGSLSEETNSSLNIVNAKFEDSGEYKCQHQQVNESEPVYLEVFSDWLLLQASAEVVMEGQPLFLRCHGWRNWDVYKVIYYKDGEALKYWYENHNISITNATVEDSGTYYCTGKVWQLDYESEPLNITVIKAPREKYWLQAQPQAEGSLAKATTAPATTRNTGRGGEEKKGSKEKEEQEERETKTPECPSHTQPLGVFLFPPKPKDTLMISRTPEVTCVVVDVSQEDPEVQFNWYVDGVEVHNAKTKPREEQFNSTYRVVSVLTVLHQDWLNGKEYKCKVSNKGLPSSIEKTISKAKGQPREPQVYTLPPSQEEMTKNQVSLTCLVKGFYPSDIAVEWESNGQPENNYKTTPPVLDSDGSFFLYSRLTVDKSRWQEGNVFSCSVMHEALHNHYTQKSLSLSLGK